European Patent Application EP 4 786 489 A1, published August 5, 2026. Title: IL-22突变体及其制备方法与应用. Applicant: 南京诺艾新生物技术有限公司. The sequence listing filed with the application follows.

SEQUENCE LISTING (7 sequences)

SEQ ID NO: 1 - protein, 146 aa, synthetic construct
APISSHCRLDKSNFQQPYITNRTFMLAKEASLADNNTDVRLIGEKLFHGVSMSERCYLMKQVLNFTLEEVLFPQSDRFQPYMQEVVPFLARLSNRLSTCHIEGDDLHIQRNVQKLKDTVKKLGESGEIKAIGELDLLFMSLRNACI

SEQ ID NO: 2 - protein, 152 aa, synthetic construct
APISSHCRLDKENFQQPYITNRTFMLAKEASLADNNTDVRLIGEKLFHGVSMSERCYLMKQVLNFTLEEVLFPQSDRFQPYMAEVVPFLAALSNALSTCHIEGDDLHIQRNVQKLKDTVKKLGESGEIKAIGELDLLFMSLRNACIHHHHHH

SEQ ID NO: 3 - protein, 377 aa, synthetic construct
APISSHCRLDKSNFQQPYITNRTFMLAKEASLADNNTDVRLIGEKLFHGVSMSERCYLMKQVLNFTLEEVLFPQSDRFQPYMQEVVPFLARLSNRLSTCHIEGDDLHIQRNVQKLKDTVKKLGESGEIKAIGELDLLFMSLRNACIRVESKYGPPCPPCPAPEFLGGPSVFLFPPKPKDTLMISRTPEVTCVVVDVSQEDPEVQFNWYVDGVEVHNAKTKPREEQFGSTYRVVSVLTVLHQDWLNGKEYKCKVSNKGLPSSIEKTISKAKGQPREPQVYTLPPSQEEMTKNQVSLTCLVKGFYPSDIAVEWESNGQPENNYKTTPPVLDSDGSFFLYSRLTVDKSRWQEGNVFSCSVMHEALHNHYTQKSLSLSLGK

SEQ ID NO: 4 - DNA, 438 bp, synthetic construct
  source 1..438: mol_type = other DNA
gctcccataagttcacactgtaggctagataagtccaacttccaacagccgtacattaccaatcgcacgtttatgctggcgaaagaagcgagcttggcggacaacaacaccgatgttcgtcttatcggcgagaagttgtttcatggtgtgagcatgtctgaacgctgctatctgatgaaacaggtgttgaatttcactctggaagaagttctgttcccgcagagcgatcgttttcaaccatacatgcaagaagtcgtgccgtttctggctcgtttatctaaccgcctgtcgacctgtcatatcgagggcgacgacctgcatatccagcgtaatgttcagaaactgaaggacaccgtaaaaaagctgggtgagagcggtgagatcaaagcaattggcgagctggatttgctgttcatgtcgctgcgtaacgcctgcatt

SEQ ID NO: 5 - DNA, 456 bp, synthetic construct
  source 1..456: mol_type = other DNA
gctcccataagttcacactgtaggctagataaggagaacttccaacaaccatacatcacgaaccgtacctttatgctggcgaaagaagctagcttggcggataacaacaccgatgttcgtctgatcggcgagaaattattccacggcgtgagcatgtctgaacgctgctatctgatgaaacaggttttgaatttcaccctcgaagaggtcctgtttccgcaaagcgatcgttttcagccgtacatggcagaagtggtgccgtttctggcggcactgtcaaatgctctgtcgacctgtcatattgaaggcgacgacctgcatatccagcgtaatgttcagaagcttaaggacactgtaaaaaagctgggtgagagcggtgagatcaaagcgattggtgagctggacttgctgttcatgtccttgcgcaacgcctgcattcatcaccatcaccaccac

SEQ ID NO: 6 - DNA, 18 bp, synthetic construct
  source 1..18: mol_type = other DNA
catcaccaccaccaccac

SEQ ID NO: 7 - protein, 33 aa, synthetic construct
MAALQKSVSSFLMGTLATSCLLLLALLVQGGAA